European Patent Application EP 4 428 142 A2, published September 11, 2024. Title: BIS-OCTAHYDROPHENANTHRENE CARBOXAMIDE DERIVATIVES AND PROTEIN CONJUGATES THEREOF. Applicant: Regeneron Pharmaceuticals, Inc. Application EP. The sequence listing filed with the application follows.

SEQUENCE LISTING (16 sequences)

SEQ ID NO: 1 - DNA, 357 bp, synthetic construct
  misc_feature 1..357: note = Synthetic
  source 1..357: mol_type = other DNA
caggtgcagctgcaggagtcgggcccaggactggtgaagccttcggagaccctgtccctcacctgcactgtcactggtggctccatcagtaggaactactggagttggatccggcagcccccagggaagggactggaatggattggatatatctattacagtgggagtatcgactacaatccctccctcaagagtcgagtcaccatatcagtagacacgtccaagaaccagttctccctgaagctgagttctatgaccgctgcggacacggccgtatactactgtgcgagagatcggtggaactggaaatacggtatggacgtctggggccaagggaccacggtcatcgtctcgtca

SEQ ID NO: 2 - protein, 119 aa, synthetic construct
  REGION 1..119: note = Synthetic
QVQLQESGPGLVKPSETLSLTCTVTGGSISRNYWSWIRQPPGKGLEWIGYIYYSGSIDYNPSLKSRVTISVDTSKNQFSLKLSSMTAADTAVYYCARDRWNWKYGMDVWGQGTTVIVSS

SEQ ID NO: 3 - DNA, 24 bp, synthetic construct
  misc_feature 1..24: note = Synthetic
  source 1..24: mol_type = other DNA
ggtggctccatcagtaggaactac

SEQ ID NO: 4 - protein, 8 aa, synthetic construct
  REGION 1..8: note = Synthetic
GGSISRNY

SEQ ID NO: 5 - DNA, 21 bp, synthetic construct
  misc_feature 1..21: note = Synthetic
  source 1..21: mol_type = other DNA
atctattacagtgggagtatc

SEQ ID NO: 6 - protein, 7 aa, synthetic construct
  REGION 1..7: note = Synthetic
IYYSGSI

SEQ ID NO: 7 - DNA, 39 bp, synthetic construct
  misc_feature 1..39: note = Synthetic
  source 1..39: mol_type = other DNA
gcgagagatcggtggaactggaaatacggtatggacgtc

SEQ ID NO: 8 - protein, 13 aa, synthetic construct
  REGION 1..13: note = Synthetic
ARDRWNWKYGMDV

SEQ ID NO: 9 - DNA, 327 bp, synthetic construct
  misc_feature 1..327: note = Synthetic
  source 1..327: mol_type = other DNA
gaaattgtgttgacgcagtctccaggcaccctgtctttgtctccaggggaaagagccaccctctcctgcagggccagtcagactgttagaaacaactacttagcctggtaccaccagaaacctggccaggctcccaggctcctcatctatggtgcatccagcagggccactggcatcccagacaggttcagtggcagtgggtctgggacagacttcactctcaccatcagcagactggagcctgaagattttacagtgtattactgtcaccagtatggtaactcaccttggacgttcggccaagggaccaaaatggaaatcaaacga

SEQ ID NO: 10 - protein, 109 aa, synthetic construct
  REGION 1..109: note = Synthetic
EIVLTQSPGTLSLSPGERATLSCRASQTVRNNYLAWYHQKPGQAPRLLIYGASSRATGIPDRFSGSGSGTDFTLTISRLEPEDFTVYYCHQYGNSPWTFGQGTKMEIKR

SEQ ID NO: 11 - DNA, 21 bp, synthetic construct
  misc_feature 1..21: note = Synthetic
  source 1..21: mol_type = other DNA
cagactgttagaaacaactac

SEQ ID NO: 12 - protein, 7 aa, synthetic construct
  REGION 1..7: note = Synthetic
QTVRNNY

SEQ ID NO: 13-14 - skipped (2 entries)

SEQ ID NO: 15 - DNA, 27 bp, synthetic construct
  misc_feature 1..27: note = Synthetic
  source 1..27: mol_type = other DNA
caccagtatggtaactcaccttggacg

SEQ ID NO: 16 - protein, 9 aa, synthetic construct
  REGION 1..9: note = Synthetic
HQYGNSPWT